European Patent Application EP 4 302 778 A1, published January 10, 2024. Title: Pharmaceutical Composition Containing Anti-TSLP Antibody. Applicant: CHIA TAI TIANQING PHARMACEUTICAL GROUP CO., LTD. Application EP22762538.1. The sequence listing filed with the application follows.

SEQUENCE LISTING (38 sequences)

SEQ ID NO: 1 - protein, 5 aa, Artificial Sequence
  VH-CDR1 for mouse, chimeric and humanized 1C5F12E9 antibodies
TYWMH

SEQ ID NO: 2 - protein, 17 aa, Artificial Sequence
  VH-CDR2 for mouse, chimeric and humanized 1C5F12E9 antibodies
VIDPSDSDTTYNQKFKG

SEQ ID NO: 3 - protein, 8 aa, Artificial Sequence
  VH-CDR3 for mouse, chimeric and humanized 1C5F12E9 antibodies
SLDGYYDY

SEQ ID NO: 4 - protein, 11 aa, Artificial Sequence
  VL-CDR1 for mouse, chimeric and humanized 1C5F12E9 antibodies
RPTENIYSYLA

SEQ ID NO: 5 - protein, 7 aa, Artificial Sequence
  VL-CDR2 for mouse, chimeric and humanized 1C5F12E9 antibodies
FARTLAE

SEQ ID NO: 6 - protein, 9 aa, Artificial Sequence
  VL-CDR3 for mouse, chimeric and humanized 1C5F12E9 antibodies
QHHYGTPWT

SEQ ID NO: 7 - protein, 117 aa, Artificial Sequence
  VH for mouse and chimeric 1C5F12E9 antibodies
QVQLQQPGTELVKPGASVKMSCKASGYTFTTYWMHWVKQRPGQGLEWIGVIDPSDSDTTYNQKFKGKATLTVDTSSSTAYMQLSSLTSEDSAVYYCTRSLDGYYDYWGQGTTLTVSS

SEQ ID NO: 8 - protein, 117 aa, Artificial Sequence
  VH for hu1C5F12E9-V1, hu1C5F12E9-V7, and hu1C5F12E9-V13
QVQLVQSGAEVKKPGASVKVSCKASGYTFTTYWMHWVRQAPGQGLEWIGVIDPSDSDTTYNQKFKGRATLTVDTSSSTAYMELSSLRSEDTAVYYCTRSLDGYYDYWGQGTLVTVSS

SEQ ID NO: 9 - protein, 117 aa, Artificial Sequence
  UNSURE (67): Xaa can be Arg or Lys
  UNSURE (68): Xaa can be Val or Ala
  UNSURE (72): Xaa can be Arg or Val
  VH for hu1C5F12E9-V2 - hu1C5F12E9-V6, hu1C5F12E9-V8 - hu1C5F12E9-V12, and hu1C5F12E9-V14 - hu1C5F12E9-V18
QVQLVQSGAEVKKPGASVKVSCKASGYTFTTYWMHWVRQAPGQGLEWMGVIDPSDSDTTYNQKFKGXXTMTXDTSTSTVYMELSSLRSEDTAVYYCTRSLDGYYDYWGQGTLVTVSS

SEQ ID NO: 10 - protein, 107 aa, Artificial Sequence
  VL for mouse and chimeric 1C5F12E9 antibodies
DIQMTQSPASLSASVGETVTITCRPTENIYSYLAWYQQKQGKSPHLLVYFARTLAEGVPSRFSGSGSGTQFSLKINSLQPEDFGIYYCQHHYGTPWTFGGGTKLEIK

SEQ ID NO: 11 - protein, 107 aa, Artificial Sequence
  UNSURE (43): Xaa can Ser or Ala
  UNSURE (48): Xaa can be Val or Ile
  VL for hu1C5F12E9-V1 - hu1C5F12E9-V18
DIQMTQSPSSLSASVGDRVTITCRPTENIYSYLAWYQQKPGKXPKLLXYFARTLAEGVPSRFSGSGSGTDFTLTISSLQPEDFATYYCQHHYGTPWTFGGGTKVEIK

SEQ ID NO: 12 - protein, 330 aa, Artificial Sequence
  Human IgG1 heavy chain constant region
ASTKGPSVFPLAPSSKSTSGGTAALGCLVKDYFPEPVTVSWNSGALTSGVHTFPAVLQSSGLYSLSSVVTVPSSSLGTQTYICNVNHKPSNTKVDKKVEPKSCDKTHTCPPCPAPELLGGPSVFLFPPKPKDTLMISRTPEVTCVVVDVSHEDPEVKFNWYVDGVEVHNAKTKPREEQYNSTYRVVSVLTVLHQDWLNGKEYKCKVSNKALPAPIEKTISKAKGQPREPQVYTLPPSREEMTKNQVSLTCLVKGFYPSDIAVEWESNGQPENNYKTTPPVLDSDGSFFLYSKLTVDKSRWQQGNVFSCSVMHEALHNHYTQKSLSLSPGK

SEQ ID NO: 13 - protein, 327 aa, Artificial Sequence
  Human IgG4 heavy chain constant region
ASTKGPSVFPLAPCSRSTSESTAALGCLVKDYFPEPVTVSWNSGALTSGVHTFPAVLQSSGLYSLSSVVTVPSSSLGTKTYTCNVDHKPSNTKVDKRVESKYGPPCPPCPAPEFLGGPSVFLFPPKPKDTLMISRTPEVTCVVVDVSQEDPEVQFNWYVDGVEVHNAKTKPREEQFNSTYRVVSVLTVLHQDWLNGKEYKCKVSNKGLPSSIEKTISKAKGQPREPQVYTLPPSQEEMTKNQVSLTCLVKGFYPSDIAVEWESNGQPENNYKTTPPVLDSDGSFFLYSRLTVDKSRWQEGNVFSCSVMHEALHNHYTQKSLSLSLGK

SEQ ID NO: 14 - protein, 107 aa, Artificial Sequence [sequence omitted]

SEQ ID NO: 15 - protein, 324 aa, Artificial Sequence
  Mouse IgG1 heavy chain constant region
AKTTPPSVYPLAPGSAAQTNSMVTLGCLVKGYFPEPVTVTWNSGSLSSGVHTFPAVLQSDLYTLSSSVTVPSSTWPSETVTCNVAHPASSTKVDKKIVPRDCGCKPCICTVPEVSSVFIFPPKPKDVLTITLTPKVTCVVVDISKDDPEVQFSWFVDDVEVHTAQTQPREEQFNSTFRSVSELPIMHQDWLNGKEFKCRVNSAAFPAPIEKTISKTKGRPKAPQVYTIPPPKEQMAKDKVSLTCMITDFFPEDITVEWQWNGQPAENYKNTQPIMDTDGSYFVYSKLNVQKSNWEAGNTFTCSVLHEGLHNHHTEKSLSHSPGK

SEQ ID NO: 16 - protein, 107 aa, Artificial Sequence
  Mouse kappa light chain constant region
RADAAPTVSIFPPSSEQLTSGGASVVCFLNNFYPKDINVKWKIDGSERQNGVLNSWTDQDSKDSTYSMSSTLTLTKDEYERHNSYTCEATHKTSTSPIVKSFNRGEC

SEQ ID NO: 17 - DNA, 351 bp, Artificial Sequence
  VH for mouse and chimeric 1C5F12E9 antibodies
caggtccaactgcagcagcctgggactgagctggtgaagcctggggcttcagtgaagatgtcctgcaaggcttctggctacaccttcaccacctactggatgcactgggtgaagcagaggcctggacaaggccttgagtggatcggagtgattgatccttctgatagtgatactacctacaatcaaaagttcaagggcaaggccacattgactgtagacacatcctccagcacagcctacatgcagctcagcagcctgacatctgaggactctgcggtctattactgtacaaggtcccttgatggttactacgactactggggccaaggcaccactctcacagtctcctca

SEQ ID NO: 18 - DNA, 351 bp, Artificial Sequence
  VH for mouse and chimeric 1C5F12E9 antibodies
caggtgcagctgcagcagcccggcaccgagctggtgaagcctggcgctagcgtgaagatgtcctgtaaggccagcggctacacattcactacatactggatgcactgggtgaagcagagacctggccagggcctggagtggatcggcgtgatcgaccccagcgactccgataccacctacaaccagaagtttaagggcaaggccaccctgacagtggatacaagctcctccacagcctacatgcagctgtccagcctgacctccgaggattccgccgtgtactactgcacaaggtccctggatggctactacgattactggggccagggcacaaccctgacagtcagcagc

SEQ ID NO: 19 - DNA, 351 bp, Artificial Sequence
  VH for hu1C5F12E9-V2, hu1C5F12E9-V8, and hu1C5F12E9-V14
caggtgcagctggtgcagagcggcgccgaggtgaagaagcctggcgcctccgtgaaggtgtcctgcaaggccagcggctacacattcaccacatactggatgcactgggtgagacaggcccccggccagggactggagtggatgggagtgatcgaccccagcgactccgacacaacctacaaccagaagttcaagggcagggtgacaatgaccagagacaccagcacaagcaccgtgtacatggagctgtcctccctgaggagcgaggacaccgccgtgtactactgcaccagatccctggacggctactacgactactggggccagggcaccctggtgacagtgtccagc

SEQ ID NO: 20 - DNA, 321 bp, Artificial Sequence
  VL for mouse and chimeric 1C5F12E9 antibodies
gacatccagatgactcagtctccagcctccctatctgcatctgtgggagaaactgtcaccatcacatgtcgaccaactgagaatatttacagttatttagcatggtatcagcagaaacagggaaaatctcctcacctcctggtctattttgcaagaaccttagcagaaggtgtgccatcaaggttcagtggcagtggatcaggcacacagttttctctgaagatcaacagcctgcagcctgaagattttgggatttattactgtcaacaccattatggtactccgtggacgttcggtggaggcaccaagctggaaatcaaa

SEQ ID NO: 21 - DNA, 321 bp, Artificial Sequence
  VL for mouse and chimeric 1C5F12E9 antibodies
gacatccagatgacccagtcccccgccagcctgtccgcctctgtgggagagaccgtgaccatcacatgcaggcccaccgagaatatctactcctacctggcctggtatcaacagaagcagggcaagagccctcacctgctggtgtacttcgccaggacactggccgagggcgtgccctctaggttcagcggcagcggctccggcacacagttttccctgaagatcaacagcctgcagcctgaggattttggcatctactactgccagcaccactacggcacaccctggacctttggcggcggcaccaagctggagatcaag

SEQ ID NO: 22 - DNA, 321 bp, Artificial Sequence
  VL for hu1C5F12E9-V7 - hu1C5F12E9-V12
gatatccagatgacacagagccccagcagcctgagcgccagcgtgggagacagggtgacaatcacatgcagacccaccgagaatatctacagctacctggcctggtatcaacagaagcctggcaaggcccccaagctgctgatctacttcgccagaaccctggccgagggcgtgccctctaggttcagcggctccggcagcggcaccgacttcacactgaccatctcctccctgcagcccgaggacttcgccacatactactgccagcaccactacggcacaccttggaccttcggcggcggcacaaaggtggagatcaag

SEQ ID NO: 23 - DNA, 993 bp, Artificial Sequence
  Human IgG1 heavy chain constant region
gctagcaccaagggcccatcggtcttccccctggcaccctcctccaagagcacctctgggggcacagcggccctgggctgcctggtcaaggactacttccccgaaccggtgacggtgtcgtggaactcaggcgccctgaccagcggcgtgcacaccttcccggctgtcctacagtcctcaggactctactccctcagcagcgtggtgaccgtgccctccagcagcttgggcacccagacctacatctgcaacgtgaatcacaagcccagcaacaccaaggtggacaagaaagttgagcccaaatcttgtgacaaaactcacacatgcccaccgtgcccagcacctgaactcctggggggaccgtcagtcttcctcttccccccaaaacccaaggacaccctcatgatctcccggacccctgaggtcacatgcgtggtggtggacgtgagccacgaagaccctgaggtcaagttcaactggtacgtggacggcgtggaggtgcataatgccaagacaaagccgcgggaggagcagtacaacagcacgtaccgtgtggtcagcgtcctcaccgtcctgcaccaggactggctgaatggcaaggagtacaagtgcaaggtctccaacaaagccctcccagcccccatcgagaaaaccatctccaaagccaaagggcagccccgagaaccacaggtgtacaccctgcccccatcccgggaggagatgaccaagaaccaggtcagcctgacctgcctggtcaaaggcttctatcccagcgacatcgccgtggagtgggagagcaatgggcagccggagaacaactacaagaccacgcctcccgtgctggactccgacggctccttcttcctctacagcaagctcaccgtggacaagagcaggtggcagcaggggaacgtcttctcatgctccgtgatgcatgaggctctgcacaaccactacacgcagaagagcctctccctgtctccgggtaaatga

SEQ ID NO: 24 - DNA, 984 bp, Artificial Sequence
  Human IgG4 heavy chain constant region
gccagcacaaagggcccttccgtgtttcccctggccccctgcagcaggagcacctctgagtccaccgccgccctgggctgtctggtgaaggactactttcccgagcccgtgaccgtgagctggaattccggcgccctgacatccggcgtgcacaccttccccgccgtgctgcagtcctccggcctgtacagcctgagctccgtggtgacagtgccttcctcctccctgggcaccaagacctacacatgtaatgtggatcacaagcccagcaacacaaaggtggataagagagtggagtccaagtacggccctccttgccctccctgtcctgccccagagttcctgggcggcccctctgtgttcctgttcccccctaagcccaaggacacactgatgatctccaggacccctgaggtgacctgcgtggtggtggacgtgagccaggaggaccctgaggtgcagttcaattggtacgtggatggcgtggaggtgcacaatgccaagacaaagcccagagaggagcagtttaattccacatacagggtggtgtccgtgctgaccgtgctgcaccaggattggctgaacggcaaggagtacaagtgtaaggtgagcaacaagggcctgccttcctccatcgagaagacaatcagcaaggccaagggccagcctagggagccccaggtgtacacactgcctcccagccaggaggagatgaccaagaaccaggtgagcctgacctgcctggtgaagggcttctaccctagcgacatcgccgtggagtgggagtccaacggccagcccgagaataactacaagacaacaccccccgtgctggattccgatggcagcttctttctgtactccaggctgaccgtggataagagcaggtggcaggagggcaatgtgttcagctgctccgtgatgcacgaggccctgcacaatcactacacccagaagagcctgtccctgagcctgggcaagtga

SEQ ID NO: 25 - DNA, 324 bp, Artificial Sequence
  Human kappa light chain constant region
cgtacggtggcggcgccatctgtcttcatcttcccgccatctgatgagcagttgaaatctggaactgcctctgttgtgtgcctgctgaataacttctatcccagagaggccaaagtacagtggaaggtggataacgccctccaatcgggtaactcccaggagagtgtcacagagcaggacagcaaggacagcacctacagcctcagcagcaccctgacgctgagcaaagcagactacgagaaacacaaagtctacgcctgcgaagtcacccatcagggcctgagctcgcccgtcacaaagagcttcaacaggggagagtgttga

SEQ ID NO: 26 - DNA, 975 bp, Artificial Sequence
  Mouse IgG1 heavy chain constant region
gccaaaacgacacccccatctgtctatccactggcccctggatctgctgcccaaactaactccatggtgaccctgggatgcctggtcaagggctatttccctgagccagtgacagtgacctggaactctggatccctgtccagcggtgtgcacaccttcccagctgtcctgcagtctgacctctacactctgagcagctcagtgactgtcccctccagcacctggcccagcgagaccgtcacctgcaacgttgcccacccggccagcagcaccaaggtggacaagaaaattgtgcccagggattgtggttgtaagccttgcatatgtacagtcccagaagtatcatctgtcttcatcttccccccaaagcccaaggatgtgctcaccattactctgactcctaaggtcacgtgtgttgtggtagacatcagcaaggatgatcccgaggtccagttcagctggtttgtagatgatgtggaggtgcacacagctcagacgcaaccccgggaggagcagttcaacagcactttccgctcagtcagtgaacttcccatcatgcaccaggactggctcaatggcaaggagttcaaatgcagggtcaacagtgcagctttccctgcccccatcgagaaaaccatctccaaaaccaaaggcagaccgaaggctccacaggtgtacaccattccacctcccaaggagcagatggccaaggataaagtcagtctgacctgcatgataacagacttcttccctgaagacattactgtggagtggcagtggaatgggcagccagcggagaactacaagaacactcagcccatcatggacacagatggctcttacttcgtctacagcaagctcaatgtgcagaagagcaactgggaggcaggaaatactttcacctgctctgtgttacatgagggcctgcacaaccaccatactgagaagagcctctcccactctcctggtaaatga

SEQ ID NO: 27 - DNA, 321 bp, Artificial Sequence
  Mouse kappa light chain constant region
cgggctgatgctgcaccaactgtatccatcttcccaccatccagtgagcagttaacatctggaggtgcctcagtcgtgtgcttcttgaacaacttctaccccaaagacatcaatgtcaagtggaagattgatggcagtgaacgacaaaatggcgtcctgaacagttggactgatcaggacagcaaagacagcacctacagcatgagcagcaccctcacgttgactaaggacgagtatgaacgacataacagctatacctgtgaggccactcacaagacatcaacttcacccattgtcaagagcttcaacaggggagagtgt

SEQ ID NO: 28 - protein, 141 aa, Artificial Sequence
  Recombinant human TSLP-his
YDFTNCDFEKIKAAYLSTISKDLITYMSGTKSTEFNNTVSCSNRPHCLTEIQSLTFNPTAGCASLAKEMFAMKTKAALAIWCPGYSETQINATQAMKKRRKRKVTTNKCLEQVSQLQGLWRRFNRPLLKQQHHHHHHHHHH

SEQ ID NO: 29 - protein, 140 aa, Artificial Sequence
  Recombinant cynomolgus monkey TSLP-his
MYDFTNCDFQKIEADYLRTISKDLITYMSGTKSTDFNNTVSCSNRPHCLTEIQSLTFNPTPRCASLAKEMFARKTKATLALWCPGYSETQINATQAMKKRRKRKVTTNKCLEQVSQLLGLWRRFIRTLLKKQLEHHHHHH

SEQ ID NO: 30 - protein, 446 aa, Artificial Sequence
  human TSLPR-Fc
GAAEGVQIQIIYFNLETVQVTWNASKYSRTNLTFHYRFNGDEAYDQCTNYLLQEGHTSGCLLDAEQRDDILYFSIRNGTHPVFTASRWMVYYLKPSSPKHVRFSWHQDAVTVTCSDLSYGDLLYEVQYRSPFDTEWQSKQENTCNVTIEGLDAEKCYSFWVRVKAMEDVYGPDTYPSDWSEVTCWQRGEIRDACAETPTPPKPKLSKDIEGRMDEPKSCDKTHTCPPCPAPELLGGPSVFLFPPKPKDTLMISRTPEVTCVVVDVSHEDPEVKFNWYVDGVEVHNAKTKPREEQYNSTYRVVSVLTVLHQDWLNGKEYKCKVSNKALPAPIEKTISKAKGQPREPQVYTLPPSREEMTKNQVSLTCLVKGFYPSDIAVEWESNGQPENNYKTTPPVLDSDGSFFLYSKLTVDKSRWQQGNVFSCSVMHEALHNHYTQKSLSLSPGK

SEQ ID NO: 31 - protein, 448 aa, Artificial Sequence
  human IL7Ra-Fc
ESGYAQNGDLEDAELDDYSFSCYSQLEVNGSQHSLTCAFEDPDVNTTNLEFEICGALVEVKCLNFRKLQEIYFIETKKFLLIGKSNICVKVGEKSLTCKKIDLTTIVKPEAPFDLSVIYREGANDFVVTFNTSHLQKKYVKVLMHDVAYRQEKDENKWTHVNLSSTKLTLLQRKLQPAAMYEIKVRSIPDHYFKGFWSEWSPSYYFRTPEINNSSGEPKSCDKTHTCPPCPAPELLGGPSVFLFPPKPKDTLMISRTPEVTCVVVDVSHEDPEVKFNWYVDGVEVHNAKTKPREEQYNSTYRVVSVLTVLHQDWLNGKEYKCKVSNKALPAPIEKTISKAKGQPREPQVYTLPPSREEMTKNQVSLTCLVKGFYPSDIAVEWESNGQPENNYKTTPPVLDSDGSFFLYSKLTVDKSRWQQGNVFSCSVMHEALHNHYTQKSLSLSPGK

SEQ ID NO: 32 - protein, 363 aa, Artificial Sequence
  human TSLP-Fc
YDFTNCDFEKIKAAYLSTISKDLITYMSGTKSTEFNNTVSCSNRPHCLTEIQSLTFNPTAGCASLAKEMFAMKTKAALAIWCPGYSETQINATQAMKKRRKRKVTTNKCLEQVSQLQGLWRRFNRPLLKQQEPKSCDKTHTCPPCPAPELLGGPSVFLFPPKPKDTLMISRTPEVTCVVVDVSHEDPEVKFNWYVDGVEVHNAKTKPREEQYNSTYRVVSVLTVLHQDWLNGKEYKCKVSNKALPAPIEKTISKAKGQPREPQVYTLPPSREEMTKNQVSLTCLVKGFYPSDIAVEWESNGQPENNYKTTPPVLDSDGSFFLYSKLTVDKSRWQQGNVFSCSVMHEALHNHYTQKSLSLSPGK

SEQ ID NO: 33 - protein, 371 aa, Homo sapiens
MGRLVLLWGAAVFLLGGWMALGQGGAAEGVQIQIIYFNLETVQVTWNASKYSRTNLTFHYRFNGDEAYDQCTNYLLQEGHTSGCLLDAEQRDDILYFSIRNGTHPVFTASRWMVYYLKPSSPKHVRFSWHQDAVTVTCSDLSYGDLLYEVQYRSPFDTEWQSKQENTCNVTIEGLDAEKCYSFWVRVKAMEDVYGPDTYPSDWSEVTCWQRGEIRDACAETPTPPKPKLSKFILISSLAILLMVSLLLLSLWKLWRVKKFLIPSVPDPKSIFPGLFEIHQGNFQEWITDTQNVAHLHKMAGAEQESGPEEPLVVQLAKTEAESPRMLDPQTEEKEASGGSLQLPHQPLQGGDVVTIGGFTFVMNDRSYVAL

SEQ ID NO: 34 - protein, 459 aa, Homo sapiens [sequence omitted]

SEQ ID NO: 35 - protein, 448 aa, Artificial Sequence
  Heavy chain of Tezepelumab
QMQLVESGGGVVQPGRSLRLSCAASGFTFRTYGMHWVRQAPGKGLEWVAVIWYDGSNKHYADSVKGRFTITRDNSKNTLNLQMNSLRAEDTAVYYCARAPQWELVHEAFDIWGQGTMVTVSSASTKGPSVFPLAPCSRSTSESTAALGCLVKDYFPEPVTVSWNSGALTSGVHTFPAVLQSSGLYSLSSVVTVPSSNFGTQTYTCNVDHKPSNTKVDKTVERKCCVECPPCPAPPVAGPSVFLFPPKPKDTLMISRTPEVTCVVVDVSHEDPEVQFNWYVDGVEVHNAKTKPREEQFNSTFRVVSVLTVVHQDWLNGKEYKCKVSNKGLPAPIEKTISKTKGQPREPQVYTLPPSREEMTKNQVSLTCLVKGFYPSDIAVEWESNGQPENNYKTTPPMLDSDGSFFLYSKLTVDKSRWQQGNVFSCSVMHEALHNHYTQKSLSLSPGK

SEQ ID NO: 36 - protein, 214 aa, Artificial Sequence
  Light chain of Tezepelumab
SYVLTQPPSVSVAPGQTARITCGGNNLGSKSVHWYQQKPGQAPVLVVYDDSDRPSWIPERFSGSNSGNTATLTISRGEAGDEADYYCQVWDSSSDHVVFGGGTKLTVLGQPKAAPSVTLFPPSSEELQANKATLVCLISDFYPGAVTVAWKADSSPVKAGVETTTPSKQSNNKYAASSYLSLTPEQWKSHRSYSCQVTHEGSTVEKTVAPTECS

SEQ ID NO: 37 - protein, 330 aa, Artificial Sequence [sequence omitted]

SEQ ID NO: 38 - DNA, 993 bp, Artificial Sequence
  Human IgG1 heavy chain constant region
gcctccaccaagggcccatcggtcttccccctggcaccctcctccaagagcacctctgggggcacagcggccctgggctgcctggtcaaggactacttccccgaaccggtgacggtgtcgtggaactcaggcgccctgaccagcggcgtgcacaccttcccggctgtcctacagtcctcaggactctactccctcagcagcgtggtgaccgtgccctccagcagcttgggcacccagacctacatctgcaacgtgaatcacaagcccagcaacaccaaggtggacaagaaagttgagcccaaatcttgtgacaaaactcacacatgcccaccgtgcccagcacctgaactcctggggggaccgtcagtcttcctcttccccccaaaacccaaggacaccctcatgatctcccggacccctgaggtcacatgcgtggtggtggacgtgagccacgaagaccctgaggtcaagttcaactggtacgtggacggcgtggaggtgcataatgccaagacaaagccgcgggaggagcagtacaacagcacgtaccgggtggtcagcgtcctcaccgtcctgcaccaggactggctgaatggcaaggagtacaagtgcaaggtctccaacaaagccctcccagcccccatcgagaaaaccatctccaaagccaaagggcagccccgagaaccacaggtgtacaccctgcccccatcccgggatgagctgaccaagaaccaggtcagcctgacctgcctggtcaaaggcttctatcccagcgacatcgccgtggagtgggagagcaatgggcagccggagaacaactacaagaccacgcctcccgtgctggactccgacggctccttcttcctctacagcaagctcaccgtggacaagagcaggtggcagcaggggaacgtcttctcatgctccgtgatgcatgaggctctgcacaaccactacacgcagaagagcctctccctgtctccgggtaaatga